European Patent Application EP 4 722 362 A1, published April 8, 2026. Title: 用于合成核苷酸链的组合物以及核苷酸链的合成方法. Applicant: 上海兆维科技发展有限公司. Application CN. The sequence listing filed with the application follows.

SEQUENCE LISTING (23 sequences)

SEQ ID NO: 1 - RNA, 49 nt, synthetic construct
  source 1..49: mol_type = other RNA
aggatgcgctaagtagcgtgcgttttagtactctggaaacagaatctac

SEQ ID NO: 2 - RNA, 48 nt, synthetic construct
  source 1..48: mol_type = other RNA
ggatgcgctaagtagcgtgcgttttagtactctggaaacagaatctac

SEQ ID NO: 3 - RNA, 47 nt, synthetic construct
  source 1..47: mol_type = other RNA
gatgcgctaagtagcgtgcgttttagtactctggaaacagaatctac

SEQ ID NO: 4 - RNA, 46 nt, synthetic construct
  source 1..46: mol_type = other RNA
atgcgctaagtagcgtgcgttttagtactctggaaacagaatctac

SEQ ID NO: 5 - RNA, 48 nt, synthetic construct
  source 1..48: mol_type = other RNA
aggatgcgctaagtagcgtgcgttttagtactctggaaacagaatcta

SEQ ID NO: 6 - RNA, 47 nt, synthetic construct
  source 1..47: mol_type = other RNA
aggatgcgctaagtagcgtgcgttttagtactctggaaacagaatct

SEQ ID NO: 7 - RNA, 46 nt, synthetic construct
  source 1..46: mol_type = other RNA
aggatgcgctaagtagcgtgcgttttagtactctggaaacagaatc

SEQ ID NO: 8 - RNA, 52 nt, synthetic construct
  source 1..52: mol_type = other RNA
taaaacaaggcaaaatgccgtgtttatctcgtcaacttgttggcgagatttt

SEQ ID NO: 9 - RNA, 51 nt, synthetic construct
  source 1..51: mol_type = other RNA
aaaacaaggcaaaatgccgtgtttatctcgtcaacttgttggcgagatttt

SEQ ID NO: 10 - RNA, 50 nt, synthetic construct
  source 1..50: mol_type = other RNA
aaacaaggcaaaatgccgtgtttatctcgtcaacttgttggcgagatttt

SEQ ID NO: 11 - RNA, 49 nt, synthetic construct
  source 1..49: mol_type = other RNA
aacaaggcaaaatgccgtgtttatctcgtcaacttgttggcgagatttt

SEQ ID NO: 12 - RNA, 51 nt, synthetic construct
  source 1..51: mol_type = other RNA
taaaacaaggcaaaatgccgtgtttatctcgtcaacttgttggcgagattt

SEQ ID NO: 13 - RNA, 50 nt, synthetic construct
  source 1..50: mol_type = other RNA
taaaacaaggcaaaatgccgtgtttatctcgtcaacttgttggcgagatt

SEQ ID NO: 14 - RNA, 49 nt, synthetic construct
  source 1..49: mol_type = other RNA
taaaacaaggcaaaatgccgtgtttatctcgtcaacttgttggcgagat

SEQ ID NO: 15 - DNA, 40 bp, synthetic construct
  source 1..40: mol_type = other DNA
tgagacctttgtcttagatgattttgttccgttttacgga

SEQ ID NO: 16 - DNA, 21 bp, synthetic construct
  source 1..21: mol_type = other DNA
ctagacctgttttgcttttgt

SEQ ID NO: 17 - RNA, 15 nt, synthetic construct
  source 1..15: mol_type = other RNA
ctagacctgttttgc

SEQ ID NO: 18 - RNA, 14 nt, synthetic construct
  source 1..14: mol_type = other RNA
tagacctgttttgc

SEQ ID NO: 19 - RNA, 13 nt, synthetic construct
  source 1..13: mol_type = other RNA
agacctgttttgc

SEQ ID NO: 20 - RNA, 12 nt, synthetic construct
  source 1..12: mol_type = other RNA
gacctgttttgc

SEQ ID NO: 21 - RNA, 14 nt, synthetic construct
  source 1..14: mol_type = other RNA
ctagacctgttttg

SEQ ID NO: 22 - RNA, 13 nt, synthetic construct
  source 1..13: mol_type = other RNA
ctagacctgtttt

SEQ ID NO: 23 - RNA, 12 nt, synthetic construct
  source 1..12: mol_type = other RNA
ctagacctgttt